European Patent Specification EP 3 864 154 B1, published December 25, 2024. Title: NUCLEIC ACID TO ACTIVATE GENE EXPRESSION AND PROTEIN PRODUCTION. Applicant: INSTITUTO DE BIOLOGIA MOLECULAR E CELULAR - IBMC. The sequence listing filed with the application follows.

SEQUENCE LISTING (1 sequence)

SEQ ID NO: 1 - DNA, 28 bp, Homo sapiens
aatttatttgtttttgccccttcccctt